European Patent Specification EP 4 489 718 B1, published March 11, 2026. Title: Method for encapsulating a hydrophobic compound, suspension of structured lipid particles according to this method, and uses of said suspension. Applicant: SEDERMA. Application EP. The sequence listing filed with the application follows.

SEQUENCE LISTING (27 sequences)

SEQ ID NO: 1 - protein, 4 aa, synthetic construct
  REGION 1..4: note = synthetic peptide
GQPR

SEQ ID NO: 2 - protein, 4 aa, synthetic construct
  REGION 1..4: note = synthetic peptide
RSRK

SEQ ID NO: 3 - protein, 4 aa, synthetic construct
  REGION 1..4: note = ARTIFICIAL SEQUENCE
KTFK

SEQ ID NO: 4 - protein, 4 aa, synthetic construct
  REGION 1..4: note = Synthetic peptide
KTAK

SEQ ID NO: 5 - protein, 4 aa, synthetic construct
  REGION 1..4: note = Synthetic peptide
KAYK

SEQ ID NO: 6 - protein, 4 aa, synthetic construct
  REGION 1..4: note = Synthetic peptide
KFYK

SEQ ID NO: 7 - protein, 4 aa, synthetic construct
  REGION 1..4: note = Artificial sequence
TKPR

SEQ ID NO: 8 - protein, 5 aa, synthetic construct
  REGION 1..5: note = synthetic peptide
KTTKS

SEQ ID NO: 9 - protein, 5 aa, synthetic construct
  REGION 1..5: note = synthetic peptide
KTSKS

SEQ ID NO: 10 - protein, 6 aa, synthetic construct
  REGION 1..6: note = Synthetic peptide
GKTTKS

SEQ ID NO: 11 - protein, 6 aa, synthetic construct
  REGION 1..6: note = synthetic peptide
VGVAPG

SEQ ID NO: 12 - protein, 4 aa, synthetic construct
  REGION 1..4: note = ARTIFICIAL SEQUENCE
  MOD_RES 1: note = amidation by a Palmitoyl chain on the N terminal end
KTFK

SEQ ID NO: 13 - protein, 4 aa, synthetic construct
  REGION 1..4: note = Synthetic peptide
  MOD_RES 1: note = amidation by a Elaidoyl chain on the N terminal end
KTAK

SEQ ID NO: 14 - protein, 4 aa, synthetic construct
  REGION 1..4: note = Synthetic peptide
  MOD_RES 1: note = amidation by a Elaidoyl chain on the N terminal end
KAYK

SEQ ID NO: 15 - protein, 4 aa, synthetic construct
  REGION 1..4: note = Synthetic peptide
  MOD_RES 1: note = amidation by a Elaidoyl chain on the N terminal end
KFYK

SEQ ID NO: 16 - protein, 4 aa, synthetic construct
  REGION 1..4: note = synthetic peptide
  MOD_RES 1: note = amidation by a Palmitoyl chain on the N terminal end
GQPR

SEQ ID NO: 17 - protein, 5 aa, synthetic construct
  REGION 1..5: note = synthetic peptide
  MOD_RES 1: note = amidation by a Palmitoyl chain on the N terminal end
KTTKS

SEQ ID NO: 18 - protein, 5 aa, synthetic construct
  REGION 1..5: note = synthetic peptide
  MOD_RES 1: note = amidation by a Palmitoyl chain on the N terminal end
KTSKS

SEQ ID NO: 19 - protein, 5 aa, synthetic construct
  REGION 1..5: note = synthetic peptide
  MOD_RES 1: note = amidation by a Palmitoyl chain on the N terminal end
  SITE 5: note = MISC_FEATURE - Xaa being either a Proline P or a Leucine L.
YGGFX

SEQ ID NO: 20 - protein, 6 aa, synthetic construct
  REGION 1..6: note = Synthetic peptide
  MOD_RES 1: note = amidation by a Palmitoyl chain on the N terminal end
  SITE 6: note = MISC_FEATURE - Xaa being Trp, Phe, Tyr, Tic, 7-hydroxy-Tic or Tpi
HLDIIX

SEQ ID NO: 21 - protein, 6 aa, synthetic construct
  REGION 1..6: note = synthetic peptide
  MOD_RES 1: note = amidation by a Palmitoyl chain on the N terminal end
GKTTKS

SEQ ID NO: 22 - protein, 6 aa, synthetic construct
  REGION 1..6: note = synthetic peptide
  MOD_RES 1: note = amidation by a Palmitoyl chain on the N terminal end
VGVAPG

SEQ ID NO: 23 - protein, 6 aa, synthetic construct
  REGION 1..6: note = synthetic peptide
  MOD_RES 1: note = Acetylation on the N-terminal end
  MOD_RES 6: note = NH2 on the C terminal end
EEMQRR

SEQ ID NO: 24 - protein, 5 aa, synthetic construct
  REGION 1..5: note = synthetic peptide
YAGFL

SEQ ID NO: 25 - protein, 4 aa, synthetic construct
  REGION 1..4: note = synthetic peptide
AHSH

SEQ ID NO: 26 - protein, 6 aa, synthetic construct
  REGION 1..6: note = synthetic peptide
SIKVAV

SEQ ID NO: 27 - protein, 6 aa, synthetic construct
  REGION 1..6: note = synthetic peptide
GPQGPQ